European Patent Specification EP 3 820 893 B1, published April 26, 2023. Title: ANTIBODIES HAVING SPECIFICITY FOR THE ORF2I PROTEIN OF HEPATITIS E VIRUS AND USES THEREOF FOR DIAGNOSTIC PURPOSES. Applicant: Inserm. The sequence listing filed with the application follows.

SEQUENCE LISTING (4 sequences)

SEQ ID NO: 1 - protein, 647 aa, Hepatitis E virus
LPMLPAPPAGQPSGRRRGRRSGGAGGGFWGDRVDSQPFALPYIHPTNPFAADIVSQSGAGTRPRQPPRPLGSAWRDQSQRPSAAPRRRSAPAGAAPLTAVSPAPDTAPVPDVDSRGAILRRQYNLSTSPLTSSVASGTNLVLYAAPLNPLLPLQDGTNTHIMATEASNYAQYRVVRATIRYRPLVPNAVGGYAISISFWPQTTTTPTSVDMNSITSTDVRILVQPGIASELVIPSERLHYRNQGWRSVETTGVAEEEATSGLVMLCIHGSPVNSYTNTPYTGALGLLDFALELEFRNLTPGNTNTRVSRYTSTARHRLRRGADGTAELTTTAATRFMKDLHFTGTNGVGEVGRGIALTLFNLADTLLGGLPTELISSAGGQLFYSRPVVSANGEPTVKLYTSVENAQQDKGITIPHDIDLGDSRVVIQDYDNQHEQDRPTPSPAPSRPFSVLRANDVLWLSLTAAEYDQATYGSSTNPMYVSDTVTFVNVATGAQAVARSLDWSKVTLDGRPLTTIQQYSKTFYVLPLRGKLSFWEAGTTRAGYPYNYNTTASDQILIENAAGHRVAISTYTTSLGAGPASISAVGVLAPHSALAVLEDTVDYPARAHTFDDFCPECRTLGLQGCAFQSTIAELQRLKTEVGKTRES

SEQ ID NO: 2 - protein, 627 aa, Hepatitis E virus
SGGAGGGFWGDRVDSQPFALPYIHPTNPFAADIVSQSGAGTRPRQPPRPLGSAWRDQSQRPSAAPRRRSAPAGAAPLTAVSPAPDTAPVPDVDSRGAILRRQYNLSTSPLTSSVASGTNLVLYAAPLNPLLPLQDGTNTHIMATEASNYAQYRVVRATIRYRPLVPNAVGGYAISISFWPQTTTTPTSVDMNSITSTDVRILVQPGIASELVIPSERLHYRNQGWRSVETTGVAEEEATSGLVMLCIHGSPVNSYTNTPYTGALGLLDFALELEFRNLTPGNTNTRVSRYTSTARHRLRRGADGTAELTTTAATRFMKDLHFTGTNGVGEVGRGIALTLFNLADTLLGGLPTELISSAGGQLFYSRPVVSANGEPTVKLYTSVENAQQDKGITIPHDIDLGDSRVVIQDYDNQHEQDRPTPSPAPSRPFSVLRANDVLWLSLTAAEYDQATYGSSTNPMYVSDTVTFVNVATGAQAVARSLDWSKVTLDGRPLTTIQQYSKTFYVLPLRGKLSFWEAGTTRAGYPYNYNTTASDQILIENAAGHRVAISTYTTSLGAGPASISAVGVLAPHSALAVLEDTVDYPARAHTFDDFCPECRTLGLQGCAFQSTIAELQRLKTEVGKTRES

SEQ ID NO: 3 - protein, 559 aa, Hepatitis E virus
SAPAGAAPLTAVSPAPDTAPVPDVDSRGAILRRQYNLSTSPLTSSVASGTNLVLYAAPLNPLLPLQDGTNTHIMATEASNYAQYRVVRATIRYRPLVPNAVGGYAISISFWPQTTTTPTSVDMNSITSTDVRILVQPGIASELVIPSERLHYRNQGWRSVETTGVAEEEATSGLVMLCIHGSPVNSYTNTPYTGALGLLDFALELEFRNLTPGNTNTRVSRYTSTARHRLRRGADGTAELTTTAATRFMKDLHFTGTNGVGEVGRGIALTLFNLADTLLGGLPTELISSAGGQLFYSRPVVSANGEPTVKLYTSVENAQQDKGITIPHDIDLGDSRVVIQDYDNQHEQDRPTPSPAPSRPFSVLRANDVLWLSLTAAEYDQATYGSSTNPMYVSDTVTFVNVATGAQAVARSLDWSKVTLDGRPLTTIQQYSKTFYVLPLRGKLSFWEAGTTRAGYPYNYNTTASDQILIENAAGHRVAISTYTTSLGAGPASISAVGVLAPHSALAVLEDTVDYPARAHTFDDFCPECRTLGLQGCAFQSTIAELQRLKTEVGKTRES

SEQ ID NO: 4 - protein, 14 aa, Hepatitis E virus
AGYPYNYNTTASDQ